European Patent Application EP 4 242 226 A1, published September 13, 2023. Title: NANOBODIES AGAINST SEVERE ACCUTE RESPIRATORY SYNDROME CORONAVIRUS 2. Applicant: CONSEJO SUPERIOR DE INVESTIGACIONES CIENTÍFICAS FUNDACIÓN CANARIA PARQUE CIENTÍFICO TECNOLÓGICO DE LA UNIVERSIDAD DE LAS PALMAS DE GRAN CANARIA. The sequence listing filed with the application follows.

SEQUENCE LISTING (45 sequences)

SEQ ID NO: 1 - protein, 10 aa, Artificial Sequence
  1.10 nanobody CDR1
GYTYSTCRKG

SEQ ID NO: 2 - protein, 9 aa, Artificial Sequence
  1.10 nanobody CDR2
SITADGATY

SEQ ID NO: 3 - protein, 11 aa, Artificial Sequence
  1.10 nanobody CDR3
SVKDFTCTFNS

SEQ ID NO: 4 - protein, 10 aa, Artificial Sequence
  1.26 nanobody CDR1
GYTWSSVCMG

SEQ ID NO: 5 - protein, 10 aa, Artificial Sequence
  1.26 nanobody CDR2
GIPSGRNRPY

SEQ ID NO: 6 - protein, 12 aa, Artificial Sequence
  1.26 nanobody CDR3
PCSAPHDPEYNY

SEQ ID NO: 7 - protein, 10 aa, Artificial Sequence
  1.28 nanobody CDR1
GLTNIRCHMA

SEQ ID NO: 8 - protein, 9 aa, Artificial Sequence
  1.28 nanobody CDR2
RITTNGVTD

SEQ ID NO: 9 - protein, 8 aa, Artificial Sequence
  1.28 nanobody CDR 3
CGFSTTTY

SEQ ID NO: 10 - protein, 10 aa, Artificial Sequence
  1.29 nanobody CDR1
GYTINTDAVA

SEQ ID NO: 11 - protein, 10 aa, Artificial Sequence
  1.29 nanobody CDR 2
VIYTGSGNTN

SEQ ID NO: 12 - protein, 13 aa, Artificial Sequence
  1.29 nanobody CDR 3
SGYYGASGYDFNN

SEQ ID NO: 13 - protein, 11 aa, Artificial Sequence
  2.1 nanobody CDR 1
FGATISSAHMG

SEQ ID NO: 14 - protein, 10 aa, Artificial Sequence
  2.1 nanobody CDR2
FRYTDGSSTY

SEQ ID NO: 15 - protein, 15 aa, Artificial Sequence
  2.1 nanobody CDR 3
SNPSWGRLVGGQYNN

SEQ ID NO: 16 - protein, 11 aa, Artificial Sequence
  2.15 nanobody CDR 1
GYASWARKCIG

SEQ ID NO: 17 - protein, 10 aa, Artificial Sequence
  2.15 nanobody CDR 2
AIFDFDGSTY

SEQ ID NO: 18 - protein, 17 aa, Artificial Sequence
  2.15 nanobody CDR 3
TVAFGTCDNWYRGRGDY

SEQ ID NO: 19 - protein, 10 aa, Artificial Sequence
  2.20 nanobody CDR 1
GYTYNNYYMG

SEQ ID NO: 20 - protein, 9 aa, Artificial Sequence
  2.20 nanobody CDR 2
AINSDGLDT

SEQ ID NO: 21 - protein, 19 aa, Artificial Sequence
  2.20 nanobody CDR 3
TGRTVYYSGYDFRLSVDDY

SEQ ID NO: 22 - protein, 119 aa, Artificial Sequence
  1.10 nanobody variable region
QVQLVESGGGSVQAGGSLRLSCAASGYTYSTCRKGWYRQAPGKERELVASITADGATYYLDSVKGRLTISQDNAKNTVYLQMNSLKPEDTAVYYCAASVKDFTCTFNSWGQGTQVTVSS

SEQ ID NO: 23 - protein, 120 aa, Artificial Sequence
  1.26 nanobody variable region
QVQLVESGGGLVQAGGSLRLSCAATGYTWSSVCMGWFRQAPGKEREGVAGIPSGRNRPYYADSVKGRFTISQDNAKNAVFLLMNSLKPEDTAIYYCAPCSAPHDPEYNYWGQGTQVTVSS

SEQ ID NO: 24 - protein, 116 aa, Artificial Sequence
  1.28 nanobody variable region
QVQLVESGGGSVQAGGSLRLSCAASGLTNIRCHMAWYRQAPGKGRELVSRITTNGVTDYADSVKERFTISRHNAENTVYLQMNSLKPEDTAVYYCAACGFSTTTYWGQGTQVTVSS

SEQ ID NO: 25 - protein, 121 aa, Artificial Sequence
  1.29 nanobody variable region
QVQLVESGGGSVQAGGSLRLSCAASGYTINTDAVAWFRQAPGKGDERVAVIYTGSGNTNYADSVKGRFTISQDNAKNTVYLQMNSLKPEDTALYYCASGYYGASGYDFNNWGQGTQVTVSS

SEQ ID NO: 26 - protein, 123 aa, Artificial Sequence
  2.1 nanobody variable region
QVQLVESGGGSVQAGGSLRLSCAAFGATISSAHMGWFRQAPGKEREGVAFRYTDGSSTYYTTSVRGRFTISQDNAKNTVYLQMNSLKPEDTAMYYCASNPSWGRLVGGQYNNWGQGTQITVSS

SEQ ID NO: 27 - protein, 125 aa, Artificial Sequence
  2.15 nanobody variable region
QVQLVESGGGSVQAGGSLKLSCAASGYASWARKCIGWFRQAPGQEREGVAAIFDFDGSTYYSDSVKGRFTISGDNAKNTVSLQMNSLLPKDTAVYYCTVAFGTCDNWYRGRGDYWGQGTQVTVSS

SEQ ID NO: 28 - protein, 127 aa, Artificial Sequence
  2.20 nanobody variable region
QVQLVESGGGSVQAGGSLRLSCAASGYTYNNYYMGWFRQAPGKEREGVAAINSDGLDTYVADSVKGRFTISRDNAKDTVHLQMNSLKPEDTAIYSCATGRTVYYSGYDFRLSVDDYWGQGTQVTVSS

SEQ ID NO: 29 - protein, 119 aa, Artificial Sequence
  humanized 1.10 nanobody variable region
EVQLVESGGGLVQPGGSLRLSCAASGYTYSTCRKGWYRQAPGKGRELVASITADGATYYLDSVKGRLTISRDNSKNTLYLQMNSLRAEDTAVYYCAASVKDFTCTFNSWGQGTQVTVSS

SEQ ID NO: 30 - protein, 120 aa, Artificial Sequence
  humanized 1.26 nanobody variable region
EVQLVESGGGLVQPGGSLRLSCAATGYTWSSVCMGWFRQAPGKGREGVAGIPSGRNRPYYADSVKGRFTISRDNAKNAVYLQMNSLRAEDTAVYYCAPCSAPHDPEYNYWGQGTQVTVSS

SEQ ID NO: 31 - protein, 121 aa, Artificial Sequence
  Humanized 1.29 nanobody variable region
EVQLVESGGGLVQPGGSLRLSCAASGYTINTDAVAWFRQAPGKGDERVAVIYTGSGNTNYADSVKGRFTISRDNAKNTVYLQMNSLRAEDTAVYYCASGYYGASGYDFNNWGQGTQVTVSS

SEQ ID NO: 32 - protein, 125 aa, Artificial Sequence
  Humanized 2.15 nanobody variable region
EVQLVESGGGLVQPGGSLKLSCAASGYASWARKCIGWFRQAPGQGREGVAAIFDFDGSTYYADSVKGRFTISRDNAKNTLYLQMNSLRAEDTAVYYCTVAFGTCDNWYRGRGDYWGQGTQVTVSS

SEQ ID NO: 33 - protein, 15 aa, Artificial Sequence
  Linker
GGGGSGGGGSGGGGS

SEQ ID NO: 34 - protein, 6 aa, Artificial Sequence
  Thrombin recognition site
LVPRGS

SEQ ID NO: 35 - DNA, 50 bp, Artificial Sequence
  VHHSfi2 primer
gtcctcgcaactgcggcccagccggccatggctcaggtgcagctggtgga

SEQ ID NO: 36 - DNA, 37 bp, Artificial Sequence
  VHHNot2 primer
ggactagtgcggccgctgaggagacggtgacctgggt

SEQ ID NO: 37 - DNA, 39 bp, Artificial Sequence
  Nb1-N2-pIg-AgeI  primer
actgcaaccggtgtacattctcaggtgcagctggtggaa

SEQ ID NO: 38 - DNA, 42 bp, Artificial Sequence
  Nb1-C5-pIg-BamHI primer
actggatccagaaccacttgccgctgaggagacggtgacctg

SEQ ID NO: 39 - DNA, 44 bp, Artificial Sequence
  Nb1-C2-pIg-BamHI primer
tcactcgaggcggatccacgcggaaccagcgctgagacggtgac

SEQ ID NO: 40 - DNA, 75 bp, Artificial Sequence
  BamHI-Nb-N-linker primer
atgggatccggaggtggcgggtccggaggtggcgggtccggaggtggcgggtcccaggtgcagctggtggagtct

SEQ ID NO: 41 - protein, 4 aa, Artificial Sequence
  Furin recognition motif
RRAR

SEQ ID NO: 42 - protein, 4 aa, Artificial Sequence
  GSAS sequence
GSAS

SEQ ID NO: 43 - protein, 9 aa, Artificial Sequence
  HA-tag
YPYDVPDYA

SEQ ID NO: 44 - protein, 125 aa, Artificial Sequence
  1.16 nanobody variable region
QVQLVESGGGSVQAGGSLRLSCAASGNTSKRKCVGWFRRAPGKEREGVTLIYTVGGSTVYADSVKGRFTISQDNAKDTVYLQMNSLKPEDSAMYYCAAESWGRQCNLETHRFTFWGQGTQVTVSS

SEQ ID NO: 45 - protein, 125 aa, Artificial Sequence
  2.11 nanobody variable region
QVQLVESGGGSVQAGGSLRLSCAASGDASNRKCVSWFRRAPGKEREGVALIFPVGSSTAYADSVKGRFTISQDSAKDTVYLQMNNLKPEDSGTYYCAAVSWGGRCNLETQTVTFWGQGTQVTVSS